European Patent Application EP 4 227 395 A1, published August 16, 2023. Title: One or more primers for HLA gene. Applicant: National Center for Global Health and Medicine H.U. Group Research Institute G.K. The sequence listing filed with the application follows.

SEQUENCE LISTING (12 sequences)

SEQ ID NO: 1 - DNA, 16 bp, Artificial Sequence
  Core sequence of forward primer for HLA-G gene
tagtgaggggcattgt

SEQ ID NO: 2 - DNA, 20 bp, Artificial Sequence
  Sequence of forward primer for HLA-G gene
gcactagtgaggggcattgt

SEQ ID NO: 3 - DNA, 17 bp, Artificial Sequence
  Core sequence of reverse primer for HLA-G gene
ctctcctctcgggaagt

SEQ ID NO: 4 - DNA, 20 bp, Artificial Sequence
  Sequence of reverse primer for HLA-G gene
gacctctcctctcgggaagt

SEQ ID NO: 5 - DNA, 16 bp, Artificial Sequence
  Core sequence of forward primer for HLA-E gene
cggcctggagaaattc

SEQ ID NO: 6 - DNA, 20 bp, Artificial Sequence
  Sequence of forward primer for HLA-E gene
ccggcctggagaaattcagt

SEQ ID NO: 7 - DNA, 16 bp, Artificial Sequence
  Core sequence of reverse primer for HLA-E gene
agaaaacagtgccacg

SEQ ID NO: 8 - DNA, 20 bp, Artificial Sequence
  Sequence of reverse primer for HLA-E gene
cccaagaaaacagtgccacg

SEQ ID NO: 9 - DNA, 15 bp, Artificial Sequence
  Core sequence of forward primer for HLA-F gene
aagagtccggggagt

SEQ ID NO: 10 - DNA, 20 bp, Artificial Sequence
  Sequence of forward primer for HLA-F gene
caaaagagtccggggagtcc

SEQ ID NO: 11 - DNA, 15 bp, Artificial Sequence
  Core sequence of reverse primer for HLA-F gene
gctcgtgaggaatgg

SEQ ID NO: 12 - DNA, 20 bp, Artificial Sequence
  Sequence of reverse primer for HLA-F gene
aaagctcgtgaggaatgggg